European Patent Application EP 4 115 902 A1, published January 11, 2023. Title: Use of CTB006 in Combination with Ponatinib. Applicant: BEIJING SINOTAU BIO-PHARMACEUTICALS TECHNOLOGY CO., LTD. The sequence listing filed with the application follows.

SEQUENCE LISTING (6 sequences)

SEQ ID NO: 1 - protein, 5 aa, Artificial Sequence
  CDR
SYFIH

SEQ ID NO: 2 - protein, 17 aa, Artificial Sequence
  CDR
WIYPGNVNTKYSEKFKG

SEQ ID NO: 3 - protein, 7 aa, Artificial Sequence
  CDR
GEAGYFD

SEQ ID NO: 4 - protein, 11 aa, Artificial Sequence
  CDR
KASQDVSTAVA

SEQ ID NO: 5 - protein, 7 aa, Artificial Sequence
  CDR
WASTRHT

SEQ ID NO: 6 - protein, 8 aa, Artificial Sequence
  CDR
QQHYRTPW